European Patent Application EP 4 403 628 A1, published July 24, 2024. Title: Novel Acetohydroxy acid synthase variant and method of producing L-isoleucine using the same. Applicant: CJ CheilJedang Corporation. The sequence listing filed with the application follows.

SEQUENCE LISTING (26 sequences)

SEQ ID NO: 1 - protein, 172 aa, Corynebacterium sp.
  REGION 1..172: note = ilvN
MANSDVTRHILSVLVQDVDGIISRVSGMFTRRAFNLVSLVSAKTETHGINRITVVVDADELNIEQITKQLNKLIPVLKVVRLDEETTIARAIMLVKVSADSTNRPQIVDAANIFRARVVDVAPDSVVIESTGTPGKLRALLDVMEPFGIRELIQSGQIALNRGPKTMAPAKI

SEQ ID NO: 2 - DNA, 519 bp, Corynebacterium sp.
  misc_feature 1..519: note = ilvN
  source 1..519: mol_type = genomic DNA
atggctaattctgacgtcacccgccacatcctgtccgtactcgttcaggacgtagacggaatcatttcccgcgtatcaggtatgttcacccgacgcgcattcaacctcgtgtccctcgtgtctgcaaagaccgaaacacacggcatcaaccgcatcacggttgttgtcgacgccgacgagctcaacattgagcagatcaccaagcagctcaacaagctgatccccgtgctcaaagtcgtgcgacttgatgaagagaccactatcgcccgcgcaatcatgctggttaaggtctctgcggacagcaccaaccgtccgcagatcgtcgacgccgcgaacatcttccgcgcccgagtcgtcgacgtggctccagactctgtggttattgaatccacaggcaccccaggcaagctccgcgcactgcttgacgtgatggaaccattcggaatccgcgaactgatccaatccggacagattgcactcaaccgcggtccgaagaccatggctccggccaagatctaa

SEQ ID NO: 3 - protein, 172 aa, synthetic construct
  REGION 1..172: note = ilvN(D17A)
MANSDVTRHILSVLVQAVDGIISRVSGMFTRRAFNLVSLVSAKTETHGINRITVVVDADELNIEQITKQLNKLIPVLKVVRLDEETTIARAIMLVKVSADSTNRPQIVDAANIFRARVVDVAPDSVVIESTGTPGKLRALLDVMEPFGIRELIQSGQIALNRGPKTMAPAKI

SEQ ID NO: 4 - protein, 172 aa, synthetic construct
  REGION 1..172: note = ilvN(D17A, A42V)
MANSDVTRHILSVLVQAVDGIISRVSGMFTRRAFNLVSLVSVKTETHGINRITVVVDADELNIEQITKQLNKLIPVLKVVRLDEETTIARAIMLVKVSADSTNRPQIVDAANIFRARVVDVAPDSVVIESTGTPGKLRALLDVMEPFGIRELIQSGQIALNRGPKTMAPAKI

SEQ ID NO: 5 - protein, 172 aa, synthetic construct
  REGION 1..172: note = ilvN(D17A, H47L)
MANSDVTRHILSVLVQAVDGIISRVSGMFTRRAFNLVSLVSAKTETLGINRITVVVDADELNIEQITKQLNKLIPVLKVVRLDEETTIARAIMLVKVSADSTNRPQIVDAANIFRARVVDVAPDSVVIESTGTPGKLRALLDVMEPFGIRELIQSGQIALNRGPKTMAPAKI

SEQ ID NO: 6 - protein, 172 aa, synthetic construct
  REGION 1..172: note = ilvN(D17A, A42V, H47L)
MANSDVTRHILSVLVQAVDGIISRVSGMFTRRAFNLVSLVSVKTETLGINRITVVVDADELNIEQITKQLNKLIPVLKVVRLDEETTIARAIMLVKVSADSTNRPQIVDAANIFRARVVDVAPDSVVIESTGTPGKLRALLDVMEPFGIRELIQSGQIALNRGPKTMAPAKI

SEQ ID NO: 7 - DNA, 30 bp, synthetic construct
  misc_feature 1..30: note = primer 9
  source 1..30: mol_type = other DNA
cgagctcggtacccatggctaattctgacg

SEQ ID NO: 8 - DNA, 30 bp, synthetic construct
  misc_feature 1..30: note = primer 10
  source 1..30: mol_type = other DNA
tagaggatccccttagatcttggccggagc

SEQ ID NO: 9 - DNA, 30 bp, synthetic construct
  misc_feature 1..30: note = primer 11
  source 1..30: mol_type = other DNA
ttcggtcttaacagacacgagggacacgag

SEQ ID NO: 10 - DNA, 30 bp, synthetic construct
  misc_feature 1..30: note = primer 12
  source 1..30: mol_type = other DNA
gtgtccctcgtgtctgttaagaccgaaaca

SEQ ID NO: 11 - DNA, 30 bp, synthetic construct
  misc_feature 1..30: note = primer 13
  source 1..30: mol_type = other DNA
cggttgatgccgagtgtttcggtctttgca

SEQ ID NO: 12 - DNA, 30 bp, synthetic construct
  misc_feature 1..30: note = primer 14
  source 1..30: mol_type = other DNA
aagaccgaaacactcggcatcaaccgcatc

SEQ ID NO: 13 - DNA, 1338 bp, synthetic construct
  misc_feature 1..1338: note = hom(R407H)
  source 1..1338: mol_type = other DNA
atgacctcagcatctgccccaagctttaaccccggcaagggtcccggctcagcagtcggaattgcccttttaggattcggaacagtcggcactgaggtgatgcgtctgatgaccgagtacggtgatgaacttgcgcaccgcattggtggcccactggaggttcgtggcattgctgtttctgatatctcaaagccacgtgaaggcgttgcacctgagctgctcactgaggacgcttttgcactcatcgagcgcgaggatgttgacatcgtcgttgaggttatcggcggcattgagtacccacgtgaggtagttctcgcagctctgaaggccggcaagtctgttgttaccgccaataaggctcttgttgcagctcactctgctgagcttgctgatgcagcggaagccgcaaacgttgacctgtacttcgaggctgctgttgcaggcgcaattccagtggttggcccactgcgtcgctccctggctggcgatcagatccagtctgtgatgggcatcgttaacggcaccaccaacttcatcttggacgccatggattccaccggcgctgactatgcagattctttggctgaggcaactcgtttgggttacgccgaagctgatccaactgcagacgtcgaaggccatgacgccgcatccaaggctgcaattttggcatccatcgctttccacacccgtgttaccgcggatgatgtgtactgcgaaggtatcagcaacatcagcgctgccgacattgaggcagcacagcaggcaggccacaccatcaagttgttggccatctgtgagaagttcaccaacaaggaaggaaagtcggctatttctgctcgcgtgcacccgactctattacctgtgtcccacccactggcgtcggtaaacaagtcctttaatgcaatctttgttgaagcagaagcagctggtcgcctgatgttctacggaaacggtgcaggtggcgcgccaaccgcgtctgctgtgcttggcgacgtcgttggtgccgcacgaaacaaggtgcacggtggccgtgctccaggtgagtccacctacgctaacctgccgatcgctgatttcggtgagaccaccactcgttaccacctcgacatggatgtggaagatcgcgtgggggttttggctgaattggctagcctgttctctgagcaaggaatctccctgcgtacaatccgacaggaagagcgcgatgatgatgcacatctgatcgtggtcacccactctgcgctggaatctgatctttcccgcaccgttgaactgctgaaggctaagcctgttgttaaggcaatcaacagtgtgatccgcctcgaaagggactaa

SEQ ID NO: 14 - DNA, 35 bp, synthetic construct
  misc_feature 1..35: note = primer 1
  source 1..35: mol_type = other DNA
tcgagctcggtaccccgcttttgcactcatcgagc

SEQ ID NO: 15 - DNA, 23 bp, synthetic construct
  misc_feature 1..23: note = primer 2
  source 1..23: mol_type = other DNA
cacgatcagatgtgcatcatcat

SEQ ID NO: 16 - DNA, 23 bp, synthetic construct
  misc_feature 1..23: note = primer 3
  source 1..23: mol_type = other DNA
atgatgatgcacatctgatcgtg

SEQ ID NO: 17 - DNA, 35 bp, synthetic construct
  misc_feature 1..35: note = primer 4
  source 1..35: mol_type = other DNA
ctctagaggatccccgagcatcttccaaaaccttg

SEQ ID NO: 18 - DNA, 1311 bp, synthetic construct
  misc_feature 1..1311: note = ilvA(T381A, F383A)
  source 1..1311: mol_type = other DNA
atgagtgaaacatacgtgtctgagaaaagtccaggagtgatggctagcggagcggagctgattcgtgccgccgacattcaaacggcgcaggcacgaatttcctccgtcattgcaccaactccattgcagtattgccctcgtctttctgaggaaaccggagcggaaatctaccttaagcgtgaggatctgcaggatgttcgttcctacaagatccgcggtgcgctgaactctggagcgcagctcactcaggagcagcgcgatgcaggtatcgttgccgcatctgcaggtaaccatgcccagggcgtggcctatgtgtgcaagtccttgggcgttcagggacgcatctatgttcctgtgcagactccaaagcaaaagcgtgaccgcatcatggttcacggcggagagtttgtctccttggtggtcactggcaataacttcgacgaagcatcggctgcagcgcatgaagatgcagagcgcaccggcgcaacgctgatcgagcctttcgatgctcgcaacaccgtcatcggtcagggtacagtggctgctgagatcttgtcgcagctgacttccatgggcaagagtgcagatcacgtgatggttccagtcggcggtggcggacttcttgcaggtgtggtcagctacatggctgatatggcacctcgcactgcgatcgttggtatcgaaccagcgggagcagcatccatgcaggctgcattgcacaatggtggaccaatcactttggagactgttgatccctttgtggacggcgcagcagtcaaacgtgtcggagatctcaactacaccatcgtggagaagaaccagggtcgcgtgcacatgatgagcgcgaccgagggcgctgtgtgtactgagatgctcgatctttaccaaaacgaaggcatcatcgcggagcctgctggcgcgctgtctatcgctgggttgaaggaaatgtcctttgcacctggttctgtcgtggtgtgcatcatctctggtggcaacaacgatgtgctgcgttatgcggaaatcgctgagcgctccttggtgcaccgcggtttgaagcactacttcttggtgaacttcccgcaaaagcctggtcagttgcgtcacttcctggaagatatcctgggaccggatgatgacatcgcgctggcagagtacctcaagcgcaacaaccgtgagaccggtactgcgttggtgggtattcacttgagtgaagcatcaggattggattctttgctggaacgtatggaggaatcggcaattgattcccgtcgcctcgagccgggcacccctgagtacgaatacttgacctaa

SEQ ID NO: 19 - DNA, 35 bp, synthetic construct
  misc_feature 1..35: note = primer 5
  source 1..35: mol_type = other DNA
tcgagctcggtacccatgagtgaaacatacgtgtc

SEQ ID NO: 20 - DNA, 39 bp, synthetic construct
  misc_feature 1..39: note = primer 6
  source 1..39: mol_type = other DNA
gcgcttgaggtactctgccagcgcgatgtcatcatccgg

SEQ ID NO: 21 - DNA, 39 bp, synthetic construct
  misc_feature 1..39: note = primer 7
  source 1..39: mol_type = other DNA
ccggatgatgacatcgcgctggcagagtacctcaagcgc

SEQ ID NO: 22 - DNA, 34 bp, synthetic construct
  misc_feature 1..34: note = primer 8
  source 1..34: mol_type = other DNA
ctctagaggatcccccgtcaccgacacctccaca

SEQ ID NO: 23 - DNA, 519 bp, synthetic construct
  misc_feature 1..519: note = ilvN(D17A)
  source 1..519: mol_type = other DNA
atggctaattctgacgtcacccgccacatcctgtccgtactcgttcaggccgtagacggaatcatttcccgcgtatcaggtatgttcacccgacgcgcattcaacctcgtgtccctcgtgtctgcaaagaccgaaacacacggcatcaaccgcatcacggttgttgtcgacgccgacgagctcaacattgagcagatcaccaagcagctcaacaagctgatccccgtgctcaaagtcgtgcgacttgatgaagagaccactatcgcccgcgcaatcatgctggttaaggtctctgcggacagcaccaaccgtccgcagatcgtcgacgccgcgaacatcttccgcgcccgagtcgtcgacgtggctccagactctgtggttattgaatccacaggcaccccaggcaagctccgcgcactgcttgacgtgatggaaccattcggaatccgcgaactgatccaatccggacagattgcactcaaccgcggtccgaagaccatggctccggccaagatctaa

SEQ ID NO: 24 - DNA, 519 bp, synthetic construct
  misc_feature 1..519: note = ilvN(D17A, A42V)
  source 1..519: mol_type = other DNA
atggctaattctgacgtcacccgccacatcctgtccgtactcgttcaggccgtagacggaatcatttcccgcgtatcaggtatgttcacccgacgcgcattcaacctcgtgtccctcgtgtctgttaagaccgaaacacacggcatcaaccgcatcacggttgttgtcgacgccgacgagctcaacattgagcagatcaccaagcagctcaacaagctgatccccgtgctcaaagtcgtgcgacttgatgaagagaccactatcgcccgcgcaatcatgctggttaaggtctctgcggacagcaccaaccgtccgcagatcgtcgacgccgcgaacatcttccgcgcccgagtcgtcgacgtggctccagactctgtggttattgaatccacaggcaccccaggcaagctccgcgcactgcttgacgtgatggaaccattcggaatccgcgaactgatccaatccggacagattgcactcaaccgcggtccgaagaccatggctccggccaagatctaa

SEQ ID NO: 25 - DNA, 519 bp, synthetic construct
  misc_feature 1..519: note = ilvN(D17A, H47L)
  source 1..519: mol_type = other DNA
atggctaattctgacgtcacccgccacatcctgtccgtactcgttcaggccgtagacggaatcatttcccgcgtatcaggtatgttcacccgacgcgcattcaacctcgtgtccctcgtgtctgcaaagaccgaaacactcggcatcaaccgcatcacggttgttgtcgacgccgacgagctcaacattgagcagatcaccaagcagctcaacaagctgatccccgtgctcaaagtcgtgcgacttgatgaagagaccactatcgcccgcgcaatcatgctggttaaggtctctgcggacagcaccaaccgtccgcagatcgtcgacgccgcgaacatcttccgcgcccgagtcgtcgacgtggctccagactctgtggttattgaatccacaggcaccccaggcaagctccgcgcactgcttgacgtgatggaaccattcggaatccgcgaactgatccaatccggacagattgcactcaaccgcggtccgaagaccatggctccggccaagatctaa

SEQ ID NO: 26 - DNA, 519 bp, synthetic construct
  misc_feature 1..519: note = ilvN(D17A, A42V, H47L)
  source 1..519: mol_type = other DNA
atggctaattctgacgtcacccgccacatcctgtccgtactcgttcaggccgtagacggaatcatttcccgcgtatcaggtatgttcacccgacgcgcattcaacctcgtgtccctcgtgtctgttaagaccgaaacactcggcatcaaccgcatcacggttgttgtcgacgccgacgagctcaacattgagcagatcaccaagcagctcaacaagctgatccccgtgctcaaagtcgtgcgacttgatgaagagaccactatcgcccgcgcaatcatgctggttaaggtctctgcggacagcaccaaccgtccgcagatcgtcgacgccgcgaacatcttccgcgcccgagtcgtcgacgtggctccagactctgtggttattgaatccacaggcaccccaggcaagctccgcgcactgcttgacgtgatggaaccattcggaatccgcgaactgatccaatccggacagattgcactcaaccgcggtccgaagaccatggctccggccaagatctaa